European Patent Application EP 4 427 804 A2, published September 11, 2024. Title: METHODS OF DIAGNOSING CANCER. Applicant: AGENCY FOR SCIENCE TECHNOLOGY AND RESEARCH. Application EP. The sequence listing filed with the application follows.

SEQUENCE LISTING (61 sequences)

SEQ ID NO: 1 - DNA, 20 bp, synthetic construct
  misc_feature 1..20: note = ABAT Primer 1
  source 1..20: mol_type = other DNA
gaggccgtgcactttttctg

SEQ ID NO: 2 - DNA, 20 bp, synthetic construct
  misc_feature 1..20: note = ABAT Primer 2
  source 1..20: mol_type = other DNA
ccagagccggatggttgtaa

SEQ ID NO: 3 - DNA, 20 bp, synthetic construct
  misc_feature 1..20: note = ACAA1 Primer 1
  source 1..20: mol_type = other DNA
acagtgttcatcgggactgc

SEQ ID NO: 4 - DNA, 21 bp, synthetic construct
  misc_feature 1..21: note = ACAA1 Primer 2
  source 1..21: mol_type = other DNA
agatattcccagggttcccca

SEQ ID NO: 5 - DNA, 20 bp, synthetic construct
  misc_feature 1..20: note = ACAA2 Primer 1
  source 1..20: mol_type = other DNA
acataacttcacgcccctgg

SEQ ID NO: 6 - DNA, 20 bp, synthetic construct
  misc_feature 1..20: note = ACAA2 Primer 2
  source 1..20: mol_type = other DNA
gaggggcaaaagcttcgttc

SEQ ID NO: 7 - DNA, 20 bp, synthetic construct
  misc_feature 1..20: note = ACADS Primer 1
  source 1..20: mol_type = other DNA
ttgccgagaaggagttggtc

SEQ ID NO: 8 - DNA, 20 bp, synthetic construct
  misc_feature 1..20: note = ACADS Primer 2
  source 1..20: mol_type = other DNA
aggtaatccaagcctgcacc

SEQ ID NO: 9 - DNA, 20 bp, synthetic construct
  misc_feature 1..20: note = ACADSB Primer 1
  source 1..20: mol_type = other DNA
ggactggcccaaggatgttt

SEQ ID NO: 10 - DNA, 20 bp, synthetic construct
  misc_feature 1..20: note = ACADSB Primer 2
  source 1..20: mol_type = other DNA
cgagcctagcagcgttgtat

SEQ ID NO: 11 - DNA, 20 bp, synthetic construct
  misc_feature 1..20: note = ALDH6A1 Primer 1
  source 1..20: mol_type = other DNA
gcgtgggcagacacatctat

SEQ ID NO: 12 - DNA, 20 bp, synthetic construct
  misc_feature 1..20: note = ALDH6A1 Primer 2
  source 1..20: mol_type = other DNA
ctcccagcatgagggatgtc

SEQ ID NO: 13 - DNA, 20 bp, synthetic construct
  misc_feature 1..20: note = AOX1 Primer 1
  source 1..20: mol_type = other DNA
tacgtgaatggccagaaggt

SEQ ID NO: 14 - DNA, 20 bp, synthetic construct
  misc_feature 1..20: note = AOX1 Primer 2
  source 1..20: mol_type = other DNA
ggatgatgcctgatcgcctt

SEQ ID NO: 15 - DNA, 20 bp, synthetic construct
  misc_feature 1..20: note = BCKDHA Primer 1
  source 1..20: mol_type = other DNA
gacctggtgtttggccagta

SEQ ID NO: 16 - DNA, 20 bp, synthetic construct
  misc_feature 1..20: note = BCKDHA Primer 2
  source 1..20: mol_type = other DNA
gccgtagtgaacaggcatct

SEQ ID NO: 17 - DNA, 20 bp, synthetic construct
  misc_feature 1..20: note = ECHS1 Primer 1
  source 1..20: mol_type = other DNA
ctcttggtgggggttgtgaa

SEQ ID NO: 18 - DNA, 20 bp, synthetic construct
  misc_feature 1..20: note = ECHS1 Primer 2
  source 1..20: mol_type = other DNA
ttgctagcgatttgccgact

SEQ ID NO: 19 - DNA, 19 bp, synthetic construct
  misc_feature 1..19: note = HIBCH Primer 1
  source 1..19: mol_type = other DNA
aggcgtcataacgctcaac

SEQ ID NO: 20 - DNA, 20 bp, synthetic construct
  misc_feature 1..20: note = HIBCH Primer 2
  source 1..20: mol_type = other DNA
tcctccggctccctttatga

SEQ ID NO: 21 - DNA, 20 bp, synthetic construct
  misc_feature 1..20: note = HMGCS2 Primer 1
  source 1..20: mol_type = other DNA
gcccaaacgtctagactccc

SEQ ID NO: 22 - DNA, 20 bp, synthetic construct
  misc_feature 1..20: note = HMGCS2 Primer 2
  source 1..20: mol_type = other DNA
ctccattagacgggacaccg

SEQ ID NO: 23 - DNA, 20 bp, synthetic construct
  misc_feature 1..20: note = MCCC1 Primer 1
  source 1..20: mol_type = other DNA
tggggtagcccgtaaatcca

SEQ ID NO: 24 - DNA, 20 bp, synthetic construct
  misc_feature 1..20: note = MCCC1 Primer 2
  source 1..20: mol_type = other DNA
gagctccttctgcactcact

SEQ ID NO: 25 - DNA, 23 bp, synthetic construct
  misc_feature 1..23: note = beta-ACTIN Primer 1
  source 1..23: mol_type = other DNA
caaggtcatccatgacaactttg

SEQ ID NO: 26 - DNA, 20 bp, synthetic construct
  misc_feature 1..20: note = beta-ACTIN Primer 2
  source 1..20: mol_type = other DNA
ggccatccacagtcttctgg

SEQ ID NO: 27 - DNA, 23 bp, synthetic construct
  misc_feature 1..23: note = GAPDH Primer 1
  source 1..23: mol_type = other DNA
caaggtcatccatgacaactttg

SEQ ID NO: 28 - DNA, 20 bp, synthetic construct
  misc_feature 1..20: note = GAPDH Primer 2
  source 1..20: mol_type = other DNA
ggccatccacagtcttctgg

SEQ ID NO: 29 - DNA, 20 bp, synthetic construct
  misc_feature 1..20: note = ABAT Primer 3
  source 1..20: mol_type = other DNA
gaggccgtgcactttttctg

SEQ ID NO: 30 - DNA, 20 bp, synthetic construct
  misc_feature 1..20: note = ABAT Primer 4
  source 1..20: mol_type = other DNA
cgcgttttgaggctgttgaa

SEQ ID NO: 31 - DNA, 20 bp, synthetic construct
  misc_feature 1..20: note = ACAA1 Primer 3
  source 1..20: mol_type = other DNA
ttacgacattggcatggcct

SEQ ID NO: 32 - DNA, 20 bp, synthetic construct
  misc_feature 1..20: note = ACAA1 Primer 4
  source 1..20: mol_type = other DNA
cagccacattctccgaggtt

SEQ ID NO: 33 - DNA, 20 bp, synthetic construct
  misc_feature 1..20: note = ACAA2 Primer 3
  source 1..20: mol_type = other DNA
ggcaaagttccaccggaaac

SEQ ID NO: 34 - DNA, 20 bp, synthetic construct
  misc_feature 1..20: note = ACAA2 Primer 4
  source 1..20: mol_type = other DNA
actggaaaccagagccacag

SEQ ID NO: 35 - DNA, 20 bp, synthetic construct
  misc_feature 1..20: note = ACADS Primer 3
  source 1..20: mol_type = other DNA
agcctttcaccaaggagtcg

SEQ ID NO: 36 - DNA, 20 bp, synthetic construct
  misc_feature 1..20: note = ACADS Primer 4
  source 1..20: mol_type = other DNA
catctcggtagtagcgctcg

SEQ ID NO: 37 - DNA, 20 bp, synthetic construct
  misc_feature 1..20: note = ACADSB Primer 3
  source 1..20: mol_type = other DNA
ggactggcccaaggatgttt

SEQ ID NO: 38 - DNA, 20 bp, synthetic construct
  misc_feature 1..20: note = ACADSB Primer 4
  source 1..20: mol_type = other DNA
ataaatggcctcccggcttc

SEQ ID NO: 39 - DNA, 20 bp, synthetic construct
  misc_feature 1..20: note = ALDH6A1 Primer 3
  source 1..20: mol_type = other DNA
agtacctggagcaaccatgc

SEQ ID NO: 40 - DNA, 20 bp, synthetic construct
  misc_feature 1..20: note = ALDH6A1 Primer 4
  source 1..20: mol_type = other DNA
cgaagatgtactctcccgcc

SEQ ID NO: 41 - DNA, 21 bp, synthetic construct
  misc_feature 1..21: note = AOX1 Primer 3
  source 1..21: mol_type = other DNA
accgtacctgaggaagaacct

SEQ ID NO: 42 - DNA, 20 bp, synthetic construct
  misc_feature 1..20: note = AOX1 Primer 4
  source 1..20: mol_type = other DNA
tgccctctactgtggtgact

SEQ ID NO: 43 - DNA, 20 bp, synthetic construct
  misc_feature 1..20: note = BCKDHA Primer 3
  source 1..20: mol_type = other DNA
caacgatgtgtttgcggtgt

SEQ ID NO: 44 - DNA, 20 bp, synthetic construct
  misc_feature 1..20: note = BCKDHA Primer 4
  source 1..20: mol_type = other DNA
ttgacctcatccaccgaacg

SEQ ID NO: 45 - DNA, 20 bp, synthetic construct
  misc_feature 1..20: note = ECHS1 Primer 3
  source 1..20: mol_type = other DNA
aggccatccaatgtgcagaa

SEQ ID NO: 46 - DNA, 20 bp, synthetic construct
  misc_feature 1..20: note = ECHS1 Primer 4
  source 1..20: mol_type = other DNA
tccacaaaggcagacatccc

SEQ ID NO: 47 - DNA, 25 bp, synthetic construct
  misc_feature 1..25: note = HIBCH Primer 3
  source 1..25: mol_type = other DNA
tggaacagattaagttctcattgac

SEQ ID NO: 48 - DNA, 20 bp, synthetic construct
  misc_feature 1..20: note = HIBCH Primer 4
  source 1..20: mol_type = other DNA
tatggtgtgctgacccttgc

SEQ ID NO: 49 - DNA, 20 bp, synthetic construct
  misc_feature 1..20: note = HMGCS2 Primer 3
  source 1..20: mol_type = other DNA
gcccaaacgtctagactccc

SEQ ID NO: 50 - DNA, 20 bp, synthetic construct
  misc_feature 1..20: note = HMGCS2 Primer 4
  source 1..20: mol_type = other DNA
cgggcatattttctgcggtg

SEQ ID NO: 51 - DNA, 20 bp, synthetic construct
  misc_feature 1..20: note = MCCC1 Primer 3
  source 1..20: mol_type = other DNA
aaggcatgtggaagtccagg

SEQ ID NO: 52 - DNA, 20 bp, synthetic construct
  misc_feature 1..20: note = MCCC1 Primer 4
  source 1..20: mol_type = other DNA
caggatcaataccaggcgct

SEQ ID NO: 53 - DNA, 23 bp, synthetic construct
  misc_feature 1..23: note = beta-ACTIN Primer 3
  source 1..23: mol_type = other DNA
caaggtcatccatgacaactttg

SEQ ID NO: 54 - DNA, 20 bp, synthetic construct
  misc_feature 1..20: note = beta-ACTIN Primer 4
  source 1..20: mol_type = other DNA
ggccatccacagtcttctga

SEQ ID NO: 55 - DNA, 23 bp, synthetic construct
  misc_feature 1..23: note = GAPDH Primer 3
  source 1..23: mol_type = other DNA
caaggtcatccatgacaactttg

SEQ ID NO: 56 - DNA, 20 bp, synthetic construct
  misc_feature 1..20: note = GAPDH Primer 4
  source 1..20: mol_type = other DNA
ggccatccacagtcttctga

SEQ ID NO: 57 - DNA, 21 bp, synthetic construct
  misc_feature 1..21: note = BCKDK shRNA1
  source 1..21: mol_type = other DNA
cgcctgtgtgagcacaagtat

SEQ ID NO: 58 - DNA, 21 bp, synthetic construct
  misc_feature 1..21: note = BCKDK shRNA2
  source 1..21: mol_type = other DNA
ggacccagacagatggactta

SEQ ID NO: 59 - DNA, 58 bp, synthetic construct
  misc_feature 1..58: note = BCKDHA shRNA1
  source 1..58: mol_type = other DNA
ccggtccttctacatgaccaactatctcgagatagttggtcatgtagaaggatttttg

SEQ ID NO: 60 - DNA, 58 bp, synthetic construct
  misc_feature 1..58: note = BCKDHA shRNA2
  source 1..58: mol_type = other DNA
ccgggcagtcacgaaagaaggtcatctcgagatgaccttctttcgtgactgctttttg

SEQ ID NO: 61 - DNA, 20 bp, synthetic construct
  misc_feature 1..20: note = Target sequence of BCKDK
  source 1..20: mol_type = other DNA
gtcggccatcgacgcggcag